European Patent Application EP 4 238 578 A1, published September 6, 2023. Title: A pharmaceutical composition. Applicant: EISAI R&D MANAGEMENT CO., LTD. The sequence listing filed with the application follows.

SEQUENCE LISTING (20 sequences)

SEQ ID NO: 1 - protein, 119 aa, Artificial Sequence
  Synthetic polypeptide
QVQLVQSGAEVKKPGASVKVSCKASGYTFTNYYIHWVKQAPGQGLEWIGWIYPGDGSPKFNERFKGRTTLTADKSTNTAYMLLSSLRSEDTAVYFCATGPTDGDYFDYWGQGTTVTVSS

SEQ ID NO: 2 - protein, 107 aa, Artificial Sequence
  Synthetic polypeptide
DIQMTQSPSSLSASVGDRVTITCRASGNIHNFLAWYQQKPGKAPKLLIYNEKTLADGVPSRFSGSGSGTDYTLTISSLQPEDFATYFCQQFWSTPYTFGGGTKVEIK

SEQ ID NO: 3 - protein, 19 aa, Artificial Sequence
  Synthetic polypeptide
MEWSWVFLFFLSVTTGVHS

SEQ ID NO: 4 - protein, 326 aa, Artificial Sequence
  Synthetic polypeptide
ASTKGPSVFPLAPCSRSTSESTAALGCLVKDYFPEPVTVSWNSGALTSGVHTFPAVLQSSGLYSLSSVVTVPSSNFGTQTYTCNVDHKPSNTKVDKTVERKCCVECPPCPAPPAAAPSVFLFPPKPKDTLMISRTPEVTCVVVDVSHEDPEVQFNWYVDGVEVHNAKTKPREEQFNSTFRVVSVLTVVHQDWLNGKEYKCKVSNKGLPAPIEKTISKTKGQPREPQVYTLPPSREEMTKNQVSLTCLVKGFYPSDIAVEWESNGQPENNYKTTPPMLDSDGSFFLYSKLTVDKSRWQQGNVFSCSVMHEALHNHYTQKSLSLSPGK

SEQ ID NO: 5 - protein, 464 aa, Artificial Sequence
  Synthetic polypeptide
MEWSWVFLFFLSVTTGVHSQVQLVQSGAEVKKPGASVKVSCKASGYTFTNYYIHWVKQAPGQGLEWIGWIYPGDGSPKFNERFKGRTTLTADKSTNTAYMLLSSLRSEDTAVYFCATGPTDGDYFDYWGQGTTVTVSSASTKGPSVFPLAPCSRSTSESTAALGCLVKDYFPEPVTVSWNSGALTSGVHTFPAVLQSSGLYSLSSVVTVPSSNFGTQTYTCNVDHKPSNTKVDKTVERKCCVECPPCPAPPAAAPSVFLFPPKPKDTLMISRTPEVTCVVVDVSHEDPEVQFNWYVDGVEVHNAKTKPREEQFNSTFRVVSVLTVVHQDWLNGKEYKCKVSNKGLPAPIEKTISKTKGQPREPQVYTLPPSREEMTKNQVSLTCLVKGFYPSDIAVEWESNGQPENNYKTTPPMLDSDGSFFLYSKLTVDKSRWQQGNVFSCSVMHEALHNHYTQKSLSLSPGK

SEQ ID NO: 6 - protein, 20 aa, Artificial Sequence
  Synthetic polypeptide
MSVPTQVLGLLLLWLTDARC

SEQ ID NO: 7 - protein, 107 aa, Artificial Sequence [sequence omitted]

SEQ ID NO: 8 - protein, 234 aa, Artificial Sequence
  Synthetic polypeptide
MSVPTQVLGLLLLWLTDARCDIQMTQSPSSLSASVGDRVTITCRASGNIHNFLAWYQQKPGKAPKLLIYNEKTLADGVPSRFSGSGSGTDYTLTISSLQPEDFATYFCQQFWSTPYTFGGGTKVEIKRTVAAPSVFIFPPSDEQLKSGTASVVCLLNNFYPREAKVQWKVDNALQSGNSQESVTEQDSKDSTYSLSSTLTLSKADYEKHKVYACEVTHQGLSSPVTKSFNRGEC

SEQ ID NO: 9 - DNA, 1417 bp, Artificial Sequence
  Synthetic oligonucleotide
aagcttgccgccaccatggaatggtcctgggtgttcctgttcttcctgtccgtgaccaccggcgtgcactcccaggtgcagctggtgcagtctggcgccgaagtgaagaaacctggcgcctccgtgaaggtgtcctgcaaggcctccggctacaccttcaccaactactacatccactgggtgaaacaggccccaggacagggcctggaatggatcggctggatctaccccggcgacggctcccccaagttcaacgagcggttcaagggccggaccaccctgaccgccgacaagtccaccaacaccgcctacatgctgctgtcctccctgcggagcgaggataccgccgtgtacttctgcgccaccggccctaccgacggcgactacttcgactactggggccagggcaccaccgtgaccgtgtcctctgcctccaccaagggcccctccgtgttccctctggccccttgctcccggtccacctctgagtctaccgccgctctgggctgcctggtcaaagactacttccccgagcctgtgacagtgtcctggaactctggcgccctgacctctggagtgcataccttccctgccgtgctgcagtcatccggcctgtactccctgtcctccgtggtgacagtgccctcctccaacttcggcacccagacctacacctgtaacgtggaccacaagccctccaacaccaaggtggacaagaccgtggaacggaagtgctgcgtggaatgccccccctgtcctgcccctcctgccgccgctccttccgtgtttctgttccccccaaagcccaaggacaccctgatgatctcccggacccccgaagtgacctgcgtggtggtggacgtgtcccacgaggaccccgaggtgcagttcaattggtacgtggacggcgtggaagtgcacaacgccaagaccaagcccagagaggaacagttcaactccaccttccgggtggtgtccgtgctgaccgtggtgcaccaggactggctgaacggcaaagagtacaagtgcaaggtctccaacaagggcctgcctgcccccatcgaaaagaccatcagcaagaccaagggccagccccgcgagccccaggtgtacacactgccccccagccgggaagagatgaccaagaaccaggtgtccctgacctgtctggtgaaaggcttctacccctccgatatcgccgtggaatgggagtccaacggacagcccgagaacaactacaagaccaccccccccatgctggactccgacggctcattcttcctgtactccaagctgacagtggacaagtcccggtggcagcagggcaacgtgttctcctgcagcgtgatgcacgaggccctgcacaaccactacacccagaagtccctgagcctgagccccggcaagtgatgaattc

SEQ ID NO: 10 - DNA, 727 bp, Artificial Sequence
  Synthetic oligonucleotide
aagcttgccgccaccatgtccgtgcccacccaggtgctgggcctgctgctgctgtggctgaccgacgccagatgcgacatccagatgacccagtccccctccagcctgtccgcctctgtgggcgacagagtgaccatcacctgtcgggcctccggcaacatccacaactttctggcctggtatcagcagaagcccggcaaggcccccaagctgctgatctacaacgaaaagaccctggccgacggcgtgccctccagattctccggctctggctccggcaccgactacaccctgaccatctccagcctgcagcccgaggacttcgccacctacttttgccagcagttctggtccaccccctacaccttcggcggaggcaccaaggtggaaatcaagcggaccgtggccgctccctccgtgttcatcttcccaccctccgacgagcagctgaagtccggcaccgcctccgtggtgtgcctgctgaacaacttctacccccgcgaggccaaggtgcagtggaaggtggacaacgccctgcagtccggcaactcccaggaatccgtcaccgagcaggactccaaggacagcacctactccctgtcctccaccctgaccctgtccaaggccgactacgagaagcacaaggtgtacgcctgcgaagtgacccaccagggcctgtccagccccgtgaccaagtccttcaaccggggcgagtgctgatgaattc

SEQ ID NO: 11 - protein, 445 aa, Artificial Sequence
  Synthetic polypeptide
QVQLVQSGAEVKKPGASVKVSCKASGYTFTNYYIHWVKQAPGQGLEWIGWIYPGDGSPKFNERFKGRTTLTADKSTNTAYMLLSSLRSEDTAVYFCATGPTDGDYFDYWGQGTTVTVSSASTKGPSVFPLAPCSRSTSESTAALGCLVKDYFPEPVTVSWNSGALTSGVHTFPAVLQSSGLYSLSSVVTVPSSNFGTQTYTCNVDHKPSNTKVDKTVERKCCVECPPCPAPPAAAPSVFLFPPKPKDTLMISRTPEVTCVVVDVSHEDPEVQFNWYVDGVEVHNAKTKPREEQFNSTFRVVSVLTVVHQDWLNGKEYKCKVSNKGLPAPIEKTISKTKGQPREPQVYTLPPSREEMTKNQVSLTCLVKGFYPSDIAVEWESNGQPENNYKTTPPMLDSDGSFFLYSKLTVDKSRWQQGNVFSCSVMHEALHNHYTQKSLSLSPGK

SEQ ID NO: 12 - protein, 214 aa, Artificial Sequence
  Synthetic polypeptide
DIQMTQSPSSLSASVGDRVTITCRASGNIHNFLAWYQQKPGKAPKLLIYNEKTLADGVPSRFSGSGSGTDYTLTISSLQPEDFATYFCQQFWSTPYTFGGGTKVEIKRTVAAPSVFIFPPSDEQLKSGTASVVCLLNNFYPREAKVQWKVDNALQSGNSQESVTEQDSKDSTYSLSSTLTLSKADYEKHKVYACEVTHQGLSSPVTKSFNRGEC

SEQ ID NO: 13 - protein, 119 aa, Artificial Sequence; identical to SEQ ID NO: 1
  Synthetic polypeptide

SEQ ID NO: 14 - protein, 107 aa, Artificial Sequence; identical to SEQ ID NO: 2
  Synthetic polypeptide

SEQ ID NO: 15 - protein, 5 aa, Artificial Sequence
  Synthetic polypeptide
NYYIH

SEQ ID NO: 16 - protein, 17 aa, Artificial Sequence
  Synthetic polypeptide
WIYPGDGSPKFNERFKG

SEQ ID NO: 17 - protein, 10 aa, Artificial Sequence
  Synthetic polypeptide
GPTDGDYFDY

SEQ ID NO: 18 - protein, 11 aa, Artificial Sequence
  Synthetic polypeptide
RASGNIHNFLA

SEQ ID NO: 19 - protein, 7 aa, Artificial Sequence
  Synthetic polypeptide
NEKTLAD

SEQ ID NO: 20 - protein, 9 aa, Artificial Sequence
  Synthetic polypeptide
QQFWSTPYT